European Patent Specification EP 3 712 265 B1, published January 10, 2024. Title: mutated AIM. Applicant: Toru Miyazaki. The sequence listing filed with the application follows.

SEQUENCE LISTING (14 sequences)

SEQ ID NO: 1 - protein, 324 aa, Homo sapiens
VRLVGGLHRCEGRVEVEQKGQWGTVCDDGWDIKDVAVLCRELGCGAASGTPSGILYEPPAEKEQKVLIQSVSCTGTEDTLAQCEQEEVYDCSHDEDAGASCENPESSFSPVPEGVRLADGPGHCKGRVEVKHQNQWYTVCQTGWSLRAAKVVCRQLGCGRAVLTQKRCNKHAYGRKPIWLSQMSCSGREATLQDCPSGPWGKNTCNHDEDTWVECEDPFDLRLVGGDNLCSGRLEVLHKGVWGSVCDDNWGEKEDQVVCKQLGCGKSLSPSFRDRKCYGPGVGRIWLDNVRCSGEEQSLEQCQHRFWGFHDCTHQEDVAVICSG

SEQ ID NO: 2 - protein, 326 aa, Mus musculus
VQLVGGAHRCEGRVEVEHNGQWGTVCDDGWDRRDVAVVCRELNCGAVIQTPRGASYQPPASEQRVLIQGVDCNGTEDTLAQCELNYDVFDCSHEEDAGAQCENPDSDLLFIPEDVRLVDGPGHCQGRVEVLHQSQWSTVCKAGWNLQVSKVVCRQLGCGRALLTYGSCNKNTQGKGPIWMGKMSCSGQEANLRSCLLSRLENNCTHGEDTWMECEDPFELKLVGGDTPCSGRLEVLHKGSWGSVCDDNWGEKEDQVVCKQLGCGKSLHPSPKTRKIYGPGAGRIWLDDVNCSGKEQSLEFCRHRLWGYHDCTHKEDVEVICTDFDV

SEQ ID NO: 3 - protein, 324 aa, Homo sapiens
VRLVGGLHRCEGRVEVEQKGQWGTVCDDGWDIKDVAVLCRELGCGAASGTPSGILYEPPAEKEQKVLIQSVSCTGTEDTLAQCEQEEVYDCSHDEDAGASCENPESSFSPVPEGVRLADGPGHCKGRVEVKHQNQWYTVCQTGWSLRAAKVVCRQLGCGRAVLTQKRSNKHAYGRKPIWLSQMSCSGREATLQDCPSGPWGKNTCNHDEDTWVECEDPFDLRLVGGDNLCSGRLEVLHKGVWGSVCDDNWGEKEDQVVCKQLGCGKSLSPSFRDRKCYGPGVGRIWLDNVRCSGEEQSLEQCQHRFWGFHDCTHQEDVAVICSG

SEQ ID NO: 4 - protein, 324 aa, Homo sapiens
VRLVGGLHRCEGRVEVEQKGQWGTVCDDGWDIKDVAVLCRELGCGAASGTPSGILYEPPAEKEQKVLIQSVSCTGTEDTLAQCEQEEVYDCSHDEDAGASCENPESSFSPVPEGVRLADGPGHCKGRVEVKHQNQWYTVCQTGWSLRAAKVVCRQLGCGRAVLTQKRCNKHAYGRKPIWLSQMSCSGREATLQDCPSGPWGKNTCNHDEDTWVECEDPFDLRLVGGDNLCSGRLEVLHKGVWGSVCDDNWGEKEDQVVCKQLGCGKSLSPSFRDRKSYGPGVGRIWLDNVRCSGEEQSLEQCQHRFWGFHDCTHQEDVAVICSG

SEQ ID NO: 5 - protein, 324 aa, Homo sapiens
VRLVGGLHRCEGRVEVEQKGQWGTVCDDGWDIKDVAVLCRELGCGAASGTPSGILYEPPAEKEQKVLIQSVSCTGTEDTLAQCEQEEVYDCSHDEDAGASCENPESSFSPVPEGVRLADGPGHCKGRVEVKHQNQWYTVCQTGWSLRAAKVVCRQLGCGRAVLTQKRSNKHAYGRKPIWLSQMSCSGREATLQDCPSGPWGKNTCNHDEDTWVECEDPFDLRLVGGDNLCSGRLEVLHKGVWGSVCDDNWGEKEDQVVCKQLGCGKSLSPSFRDRKSYGPGVGRIWLDNVRCSGEEQSLEQCQHRFWGFHDCTHQEDVAVICSG

SEQ ID NO: 6 - protein, 326 aa, Mus musculus
VQLVGGAHRCEGRVEVEHNGQWGTVCDDGWDRRDVAVVCRELNCGAVIQTPRGASYQPPASEQRVLIQGVDCNGTEDTLAQCELNYDVFDCSHEEDAGAQCENPDSDLLFIPEDVRLVDGPGHCQGRVEVLHQSQWSTVCKAGWNLQVSKVVCRQLGCGRALLTYGSSNKNTQGKGPIWMGKMSCSGQEANLRSCLLSRLENNCTHGEDTWMECEDPFELKLVGGDTPCSGRLEVLHKGSWGSVCDDNWGEKEDQVVCKQLGCGKSLHPSPKTRKIYGPGAGRIWLDDVNCSGKEQSLEFCRHRLWGYHDCTHKEDVEVICTDFDV

SEQ ID NO: 7 - protein, 23 aa, Homo sapiens
MALLFSLILAICTRPGFLASPSG

SEQ ID NO: 8 - protein, 26 aa, Mus musculus
MAPLFNLMLAILSIFVGSCFSESPTK

SEQ ID NO: 9 - DNA, 1044 bp, Homo sapiens
atggctctgctcttcagcctcatcctcgccatctgcaccagacccggcttcctcgccagccccagcggagtgagactggtcggaggcctgcacagatgtgaaggccgcgtcgaggtggagcagaagggccagtggggcaccgtctgcgacgacggctgggacatcaaggacgtggctgtcctctgccgcgagctgggatgcggtgctgccagcggcacgcccagcggcatcctgtacgagcctcccgcagagaaggagcagaaggtcctgatccagagcgtcagctgcacaggcaccgaggacacactggctcagtgtgagcaggaggaagtctacgactgtagccacgacgaggacgctggcgcatcctgcgagaaccccgagagctccttcagccccgtgcccgagggcgtcagactggctgacggccctggccactgcaagggcagagtcgaggtgaagcaccagaaccagtggtacaccgtgtgccagaccggctggagcctcagagccgcaaaggtcgtctgccggcagctgggctgtggcagggctgtactgactcagaagcgctgcaacaagcacgcctacggccgcaagcccatctggctcagccagatgagctgcagcggccgcgaggcaaccctgcaggactgccccagcggcccttggggcaagaacacctgcaaccatgacgaggacacgtgggtcgagtgtgaagatcccttcgacttgcgcctcgtcggaggagacaacctctgcagcggccgcctcgaggtgctgcacaagggcgtctggggcagcgtctgcgacgacaactggggcgagaaggaggaccaggtggtatgcaagcaactgggctgtggcaagtccctcagccccagcttccgcgaccgcaagtgctacggtcccggcgtcggcagaatctggctggacaacgtccgctgcagcggcgaggagcagagcctcgagcagtgccagcaccgcttctggggcttccacgactgcacccaccaggaggacgtcgctgtcatctgcagcggctag

SEQ ID NO: 10 - DNA, 1059 bp, Mus musculus
atggctccattgttcaacttgatgctggccatcttgagcatttttgttggatcgtgtttttcagagtctccaaccaaagtgcagctagtgggaggtgcccaccgctgtgaagggcgagtggaggtggaacacaatggccagtgggggactgtgtgtgatgatggctgggaccggcgtgatgtggctgtggtgtgccgagagctcaattgtggagcagtcatccaaaccccgcgtggcgcatcatatcagccaccagcatcagagcaaagagttcttattcaaggggttgactgcaacggaacggaagacacgttggctcaatgtgagctaaattacgatgtttttgactgctcacatgaagaagatgctggggcacagtgtgagaacccagacagtgacctcctcttcattccagaggatgtgcgtctagtagatggcccggggcactgccagggtcgagtggaggtgctccaccagtcccagtggagcactgtgtgtaaagcaggctggaacttacaggtctcaaaggtggtgtgcaggcagctcgggtgtgggcgggcattactgacctacggaagctgcaacaagaatactcagggcaaaggacccatctggatgggcaagatgtcgtgttctggacaagaagcaaaccttcggtcttgccttttgagtcgtttggagaacaactgtacccatggcgaggacacatggatggaatgtgaagatccttttgagctgaagctggtgggaggagacaccccctgctctgggaggttggaggtgctgcacaagggttcctggggctccgtctgtgatgacaactggggagaaaaggaggaccaagtggtctgcaagcaactgggttgtgggaagtccctccatccatcccccaaaacccggaaaatctatgggcctggggcaggccgcatctggctggatgacgtcaactgctcagggaaggaacagtctctggagttctgccggcacaggttgtgggggtaccacgactgtacccacaaggaagatgtggaggtgatctgcacagactttgatgtgtga

SEQ ID NO: 11 - DNA, 1044 bp, Homo sapiens
atggctctgctcttcagcctcatcctcgccatctgcaccagacccggcttcctcgccagccccagcggagtgagactggtcggaggcctgcacagatgtgaaggccgcgtcgaggtggagcagaagggccagtggggcaccgtctgcgacgacggctgggacatcaaggacgtggctgtcctctgccgcgagctgggatgcggtgctgccagcggcacgcccagcggcatcctgtacgagcctcccgcagagaaggagcagaaggtcctgatccagagcgtcagctgcacaggcaccgaggacacactggctcagtgtgagcaggaggaagtctacgactgtagccacgacgaggacgctggcgcatcctgcgagaaccccgagagctccttcagccccgtgcccgagggcgtcagactggctgacggccctggccactgcaagggcagagtcgaggtgaagcaccagaaccagtggtacaccgtgtgccagaccggctggagcctcagagccgcaaaggtcgtctgccggcagctgggctgtggcagggctgtactgactcagaagcgctccaacaagcacgcctacggccgcaagcccatctggctcagccagatgagctgcagcggccgcgaggcaaccctgcaggactgccccagcggcccttggggcaagaacacctgcaaccatgacgaggacacgtgggtcgagtgtgaagatcccttcgacttgcgcctcgtcggaggagacaacctctgcagcggccgcctcgaggtgctgcacaagggcgtctggggcagcgtctgcgacgacaactggggcgagaaggaggaccaggtggtatgcaagcaactgggctgtggcaagtccctcagccccagcttccgcgaccgcaagtgctacggtcccggcgtcggcagaatctggctggacaacgtccgctgcagcggcgaggagcagagcctcgagcagtgccagcaccgcttctggggcttccacgactgcacccaccaggaggacgtcgctgtcatctgcagcggctag

SEQ ID NO: 12 - DNA, 1044 bp, Homo sapiens
atggctctgctcttcagcctcatcctcgccatctgcaccagacccggcttcctcgccagccccagcggagtgagactggtcggaggcctgcacagatgtgaaggccgcgtcgaggtggagcagaagggccagtggggcaccgtctgcgacgacggctgggacatcaaggacgtggctgtcctctgccgcgagctgggatgcggtgctgccagcggcacgcccagcggcatcctgtacgagcctcccgcagagaaggagcagaaggtcctgatccagagcgtcagctgcacaggcaccgaggacacactggctcagtgtgagcaggaggaagtctacgactgtagccacgacgaggacgctggcgcatcctgcgagaaccccgagagctccttcagccccgtgcccgagggcgtcagactggctgacggccctggccactgcaagggcagagtcgaggtgaagcaccagaaccagtggtacaccgtgtgccagaccggctggagcctcagagccgcaaaggtcgtctgccggcagctgggctgtggcagggctgtactgactcagaagcgctgcaacaagcacgcctacggccgcaagcccatctggctcagccagatgagctgcagcggccgcgaggcaaccctgcaggactgccccagcggcccttggggcaagaacacctgcaaccatgacgaggacacgtgggtcgagtgtgaagatcccttcgacttgcgcctcgtcggaggagacaacctctgcagcggccgcctcgaggtgctgcacaagggcgtctggggcagcgtctgcgacgacaactggggcgagaaggaggaccaggtggtatgcaagcaactgggctgtggcaagtccctcagccccagcttccgcgaccgcaagtcctacggtcccggcgtcggcagaatctggctggacaacgtccgctgcagcggcgaggagcagagcctcgagcagtgccagcaccgcttctggggcttccacgactgcacccaccaggaggacgtcgctgtcatctgcagcggctag

SEQ ID NO: 13 - DNA, 1044 bp, Homo sapiens
atggctctgctcttcagcctcatcctcgccatctgcaccagacccggcttcctcgccagccccagcggagtgagactggtcggaggcctgcacagatgtgaaggccgcgtcgaggtggagcagaagggccagtggggcaccgtctgcgacgacggctgggacatcaaggacgtggctgtcctctgccgcgagctgggatgcggtgctgccagcggcacgcccagcggcatcctgtacgagcctcccgcagagaaggagcagaaggtcctgatccagagcgtcagctgcacaggcaccgaggacacactggctcagtgtgagcaggaggaagtctacgactgtagccacgacgaggacgctggcgcatcctgcgagaaccccgagagctccttcagccccgtgcccgagggcgtcagactggctgacggccctggccactgcaagggcagagtcgaggtgaagcaccagaaccagtggtacaccgtgtgccagaccggctggagcctcagagccgcaaaggtcgtctgccggcagctgggctgtggcagggctgtactgactcagaagcgctccaacaagcacgcctacggccgcaagcccatctggctcagccagatgagctgcagcggccgcgaggcaaccctgcaggactgccccagcggcccttggggcaagaacacctgcaaccatgacgaggacacgtgggtcgagtgtgaagatcccttcgacttgcgcctcgtcggaggagacaacctctgcagcggccgcctcgaggtgctgcacaagggcgtctggggcagcgtctgcgacgacaactggggcgagaaggaggaccaggtggtatgcaagcaactgggctgtggcaagtccctcagccccagcttccgcgaccgcaagtcctacggtcccggcgtcggcagaatctggctggacaacgtccgctgcagcggcgaggagcagagcctcgagcagtgccagcaccgcttctggggcttccacgactgcacccaccaggaggacgtcgctgtcatctgcagcggctag

SEQ ID NO: 14 - DNA, 1059 bp, Mus musculus
atggctccattgttcaacttgatgctggccatcttgagcatttttgttggatcgtgtttttcagagtctccaaccaaagtgcagctagtgggaggtgcccaccgctgtgaagggcgagtggaggtggaacacaatggccagtgggggactgtgtgtgatgatggctgggaccggcgtgatgtggctgtggtgtgccgagagctcaattgtggagcagtcatccaaaccccgcgtggcgcatcatatcagccaccagcatcagagcaaagagttcttattcaaggggttgactgcaacggaacggaagacacgttggctcaatgtgagctaaattacgatgtttttgactgctcacatgaagaagatgctggggcacagtgtgagaacccagacagtgacctcctcttcattccagaggatgtgcgtctagtagatggcccggggcactgccagggtcgagtggaggtgctccaccagtcccagtggagcactgtgtgtaaagcaggctggaacttacaggtctcaaaggtggtgtgcaggcagctcgggtgtgggcgggcattactgacctacggaagctccaacaagaatactcagggcaaaggacccatctggatgggcaagatgtcgtgttctggacaagaagcaaaccttcggtcttgccttttgagtcgtttggagaacaactgtacccatggcgaggacacatggatggaatgtgaagatccttttgagctgaagctggtgggaggagacaccccctgctctgggaggttggaggtgctgcacaagggttcctggggctccgtctgtgatgacaactggggagaaaaggaggaccaagtggtctgcaagcaactgggttgtgggaagtccctccatccatcccccaaaacccggaaaatctatgggcctggggcaggccgcatctggctggatgacgtcaactgctcagggaaggaacagtctctggagttctgccggcacaggttgtgggggtaccacgactgtacccacaaggaagatgtggaggtgatctgcacagactttgatgtgtga